European Patent Application EP 4 640 704 A1, published October 29, 2025. Title: ANTIBODIES SPECIFIC TO HUMAN HMGI-C ANTIGEN AND USE THEREOF. Applicant: PeriCard Check GmbH. Application EP. The sequence listing filed with the application follows.

SEQUENCE LISTING (59 sequences)

SEQ ID NO: 1 - protein, 440 aa, synthetic construct
EVQLQQSGPELVKPGASVRISCKASGYSFTGHYMHWVKQSPENSLEWIGEINPTTGGITYNQKFKGKATLTVDKSSITAYMHLKSLTSEDSAVYYCTGGGDHFDYWGQGTTLTVSSAKTTPPSVYPLAPGSAAQTNSMVTLGCLVKGYFPEPVTVTWNSGSLSSGVHTFPAVLQSDLYTLSSSVTVPSSTWPSETVTCNVAHPASSTKVDKKIVPRDCGCKPCICTVPEVSSVFIFPPKPKDVLTITLTPKVTCVVVDISKDDPEVQFSWFVDDVEVHTAQTQPREEQFNSTFRSVSELPIMHQDWLNGKEFKCRVNSAAFPAPIEKTISKTKGRPKAPQVYTIPPPKEQMAKDKVSLTCMITDFFPEDITVEWQWNGQPAENYKNTQPIMDTDGSYFVYSKLNVQKSNWEAGNTFTCSVLHEGLHNHHTEKSLSHSPGK

SEQ ID NO: 2 - protein, 8 aa, synthetic construct
GYSFTGHY

SEQ ID NO: 3 - protein, 8 aa, synthetic construct
INPTTGGI

SEQ ID NO: 4 - protein, 9 aa, synthetic construct
TGGGDHFDY

SEQ ID NO: 5 - DNA, 1320 bp, synthetic construct
  source 1..1320: mol_type = other DNA
gaggtccaactgcagcagtctggacctgagctggtgaagcctggggcttcagtgaggatatcctgcaaggcttctggttactcattcactggccactacatgcactgggtgaagcaaagtcctgaaaatagtcttgagtggattggagagattaatcctaccactgggggtattacctacaaccagaagttcaagggcaaggccacattaactgtagataaatcctccatcacagcctacatgcacctcaagagcctgacatctgaagactctgcagtctattactgtacaggcgggggggaccactttgactactggggccaaggcaccactctcacagtctcctcagccaaaacgacacccccatctgtctatccactggcccctggatctgctgcccaaactaactccatggtgaccctgggatgcctggtcaagggctatttccctgagccagtgacagtgacctggaactctggatccctgtccagcggtgtgcacaccttcccagctgtcctgcagtctgacctctacactctgagcagctcagtgactgtcccctccagcacctggcccagcgagaccgtcacctgcaacgttgcccacccggccagcagcaccaaggtggacaagaaaattgtgcccagggattgtggttgtaagccttgcatatgtacagtcccagaagtatcatctgtcttcatcttccccccaaagcccaaggatgtgctcaccattactctgactcctaaggtcacgtgtgttgtggtagacatcagcaaggatgatcccgaggtccagttcagctggtttgtagatgatgtggaggtgcacacagctcagacgcaaccccgggaggagcagttcaacagcactttccgctcagtcagtgaacttcccatcatgcaccaggactggctcaatggcaaggagttcaaatgcagggtcaacagtgcagctttccctgcccccatcgagaaaaccatctccaaaaccaaaggcagaccgaaggctccacaggtgtacaccattccacctcccaaggagcagatggccaaggataaagtcagtctgacctgcatgataacagacttcttccctgaagacattactgtggagtggcagtggaatgggcagccagcggagaactacaagaacactcagcccatcatggacacagatggctcttacttcgtctacagcaagctcaatgtgcagaagagcaactgggaggcaggaaatactttcacctgctctgtgttacatgagggcctgcacaaccaccatactgagaagagcctctcccactctcctggtaaa

SEQ ID NO: 6 - protein, 219 aa, synthetic construct
DVSMTQSPLSLPVSLGDQVSISCRSSQSILHSNGNTYLEWFLQRPGQSPKLLIYKVSNRFSGVPDRFSGSGSGTDFTLKISRVEAEDLGVYYCFQGSHDPPTFGGGTKLEIKRADAAPTVSIFPPSSEQLTSGGASVVCFLNNFYPKDINVKWKIDGSERQNGVLNSWTDQDSKDSTYSMSSTLTLTKDEYERHNSYTCEATHKTSTSPIVKSFNRNEC

SEQ ID NO: 7 - protein, 11 aa, synthetic construct
QSILHSNGNTY

SEQ ID NO: 8 - skipped

SEQ ID NO: 9 - protein, 9 aa, synthetic construct
FQGSHDPPT

SEQ ID NO: 10 - DNA, 657 bp, synthetic construct
  source 1..657: mol_type = other DNA
gatgtttcgatgacccaaagtccactctccctgcctgtcagtcttggagatcaagtctccatctcttgcagatccagtcagagcattttacatagtaacggaaacacctatttagaatggttcctgcagagaccaggccagtctccaaagctcctgatctacaaagtttccaaccgattttctggggtcccagacaggttcagtggcagtggatcagggacagatttcacactcaagatcagcagagtggaggctgaggatctgggagtttattactgctttcaaggttcacatgatcctccgacgttcggtggaggcaccaagctggaaatcaaacgggctgatgctgcaccaactgtatccatcttcccaccatccagtgagcagttaacatctggaggtgcctcagtcgtgtgcttcttgaacaacttctaccccaaagacatcaatgtcaagtggaagattgatggcagtgaacgacaaaatggcgtcctgaacagttggactgatcaggacagcaaagacagcacctacagcatgagcagcaccctcacgttgaccaaggacgagtatgaacgacataacagctatacctgtgaggccactcacaagacatcaacttcacccattgtcaagagcttcaacaggaatgagtgt

SEQ ID NO: 11 - protein, 454 aa, synthetic construct
QIQLVQSGPELKKPGETVKISCKASGYTFTNYGMNWVKQAPGKDLKWMGWINTYTGEPTYADDFKGRFVFSLETSASTAYLQINNLNNKDTATYFCAREGRLLYFHVWGAGTTVTVSSAKTTPPSVYPLAPGCGDTTGSSVTLGCLVKGYFPESVTVTWNSGSLSSSVHTFPALLQSGLYTMSSSVTVPSSTWPSQTVTCSVAHPASSTTVDKKLEPSGPISTINPCPPCKECHKCPAPNLEGGPSVFIFPPNIKDVLMISLTPKVTCVVVDVSEDDPDVRISWFVNNVEVHTAQTQTHREDYNSTIRVVSALPIQHQDWMSGKEFKCKVNNKDLPSPIERTISKIKGLVRAPQVYILPPPAEQLSRKDVSLTCLVVGFNPGDISVEWTSNGHTEENYKDTAPVLDSDGSYFIYSKLDIKTSKWEKTDSFSCNVRHEGLKNYYLKKTISRSPGK

SEQ ID NO: 12 - protein, 8 aa, synthetic construct
GYTFTNYG

SEQ ID NO: 13 - protein, 8 aa, synthetic construct
INTYTGEP

SEQ ID NO: 14 - protein, 11 aa, synthetic construct
AREGRLLYFHV

SEQ ID NO: 15 - DNA, 1362 bp, synthetic construct
  source 1..1362: mol_type = other DNA
cagatccagttggtgcagtctggacctgagctgaagaagcctggagagacagtcaagatctcctgcaaggcttctgggtataccttcacaaactatggaatgaactgggtgaagcaggctccaggaaaggatttaaagtggatgggctggataaacacctacactggagagccaacatatgctgatgacttcaagggacggtttgtcttctctttggaaacctctgccagcactgcctatttgcagatcaacaacctcaacaataaagacacggctacatatttctgtgcaagagaggggaggctactatatttccatgtctggggcgcagggaccacggtcaccgtctcctcagctaaaacaacacccccatcagtctatccactggcccctgggtgtggagatacaactggttcctctgtgactctgggatgcctggtcaagggctacttccctgagtcagtgactgtgacttggaactctggatccctgtccagcagtgtgcacaccttcccagctctcctgcagtctggactctacactatgagcagctcagtgactgtcccctccagcacctggccaagtcagaccgtcacctgcagcgttgctcacccagccagcagcaccacggtggacaaaaaacttgagcccagcgggcccatttcaacaatcaacccctgtcctccatgcaaggagtgtcacaaatgcccagctcctaacctcgagggtggaccatccgtcttcatcttccctccaaatatcaaggatgtactcatgatctccctgacacccaaggtcacgtgtgtggtggtggatgtgagcgaggatgacccagacgtccggatcagctggtttgtgaacaacgtggaagtacacacagctcagacacaaacccatagagaggattacaacagtactatccgggtggtcagtgccctccccatccagcaccaggactggatgagtggcaaggagttcaaatgcaaggtcaacaacaaagacctcccatcacccatcgagagaaccatctcaaaaattaaagggctagtcagagctccacaagtatacatcttgccgccaccagcagagcagttgtccaggaaagatgtcagtctcacttgcctggtcgtgggcttcaaccctggagacatcagtgtggagtggaccagcaatgggcatactgaggagaactacaaggacaccgcaccagtcctggactctgacggttcttacttcatatacagcaagctcgatataaaaacaagcaagtgggagaaaacagattccttctcatgcaacgtgagacacgagggtctgaaaaattactacctgaagaagaccatctcccggtctccgggtaaa

SEQ ID NO: 16 - protein, 219 aa, synthetic construct
DVLMTQTPLSLPVSLGDQASISCRSSQRIVHSNGNTYLEWYLQKPGQSPKLLIYKVSNRFSGVPDRFSGSGSGTDFTLKITRVEAEDLGVYYCFQGSHVPYTFGGGTKLEIKRADAAPTVSIFPPSSEQLTSGGASVVCFLNNFYPKDINVKWKIDGSERQNGVLNSWTDQDSKDSTYSMSSTLTLTKDEYERHNSYTCEATHKTSTSPIVKSFNRNEC

SEQ ID NO: 17 - protein, 11 aa, synthetic construct
QRIVHSNGNTY

SEQ ID NO: 18 - skipped

SEQ ID NO: 19 - protein, 9 aa, synthetic construct
FQGSHVPYT

SEQ ID NO: 20 - DNA, 657 bp, synthetic construct
  source 1..657: mol_type = other DNA
gatgttttgatgacccaaactccactctccctgcctgtcagtcttggagatcaagcctccatctcttgcagatctagtcagcgcattgtacatagtaatggaaacacgtatttagaatggtacctgcagaaaccaggccagtctccaaagctcctgatctacaaagtttccaaccgattttctggggtcccagacaggttcagtggcagtggatcagggacagatttcacactcaagatcaccagagtggaggctgaggatctgggagtttattactgctttcaaggttcacatgttccgtacacattcggaggggggaccaagctggaaataaaacgggctgatgctgcaccaactgtatccatcttcccaccatccagtgagcagttaacatctggaggtgcctcagtcgtgtgcttcttgaacaacttctaccccaaagacatcaatgtcaagtggaagattgatggcagtgaacgacaaaatggcgtcctgaacagttggactgatcaggacagcaaagacagcacctacagcatgagcagcaccctcacgttgaccaaggacgagtatgaacgacataacagctatacctgtgaggccactcacaagacatcaacttcacccattgtcaagagcttcaacaggaatgagtgt

SEQ ID NO: 21 - protein, 456 aa, synthetic construct
EVKLEQSGPELKKPGETVKISCMASGYTFTDYSIHWVRQAPGKGLKWMAWINTETGETTYADDFKGRFAFSLETSASTAYLQINNLENEDTATYYCARWGYDYYDGMDYWGQGTSVTVSSAKTTPPSVYPLAPGCGDTTGSSVTLGCLVKGYFPESVTVTWNSGSLSSSVHTFPALLQSGLYTMSSSVTVPSSTWPSQTVTCSVAHPASSTTVDKKLEPSGPISTINPCPPCKECHKCPAPNLEGGPSVFIFPPNIKDVLMISLTPKVTCVVVDVSEDDPDVRISWFVNNVEVHTAQTQTHREDYNSTIRVVSALPIQHQDWMSGKEFKCKVNNKDLPSPIERTISKIKGLVRAPQVYILPPPAEQLSRKDVSLTCLVVGFNPGDISVEWTSNGHTEENYKDTAPVLDSDGSYFIYSKLDIKTSKWEKTDSFSCNVRHEGLKNYYLKKTISRSPGK

SEQ ID NO: 22 - protein, 8 aa, synthetic construct
GYTFTDYS

SEQ ID NO: 23 - protein, 8 aa, synthetic construct
INTETGET

SEQ ID NO: 24 - protein, 13 aa, synthetic construct
ARWGYDYYDGMDY

SEQ ID NO: 25 - DNA, 1368 bp, synthetic construct
  source 1..1368: mol_type = other DNA
gaggtgaagctggagcagtcaggacctgagctgaagaagcctggagagacagtcaagatctcctgcatggcttctggttacaccttcacagactattcaattcactgggtgaggcaggctccaggaaagggtttaaagtggatggcctggataaacactgagactggtgagacaacatatgcagatgacttcaagggacggtttgccttctctttggaaacctctgccagcacggcctatttgcagatcaacaacctcgaaaatgaggacacggctacatattactgtgctaggtgggggtatgattactacgatggtatggactactggggtcaaggaacttcagtcaccgtctcctcagctaaaacaacacccccatcagtctatccactggcccctgggtgtggagatacaactggttcctctgtgactctgggatgcctggtcaagggctacttccctgagtcagtgactgtgacttggaactctggatccctgtccagcagtgtgcacaccttcccagctctcctgcagtctggactctacactatgagcagctcagtgactgtcccctccagcacctggccaagtcagaccgtcacctgcagcgttgctcacccagccagcagcaccacggtggacaaaaaacttgagcccagcgggcccatttcaacaatcaacccctgtcctccatgcaaggagtgtcacaaatgcccagctcctaacctcgagggtggaccatccgtcttcatcttccctccaaatatcaaggatgtactcatgatctccctgacacccaaggtcacgtgtgtggtggtggatgtgagcgaggatgacccagacgtccggatcagctggtttgtgaacaacgtggaagtacacacagctcagacacaaacccatagagaggattacaacagtactatccgggtggtcagtgccctccccatccagcaccaggactggatgagtggcaaggagttcaaatgcaaggtcaacaacaaagacctcccatcacccatcgagagaaccatctcaaaaattaaagggctagtcagagctccacaagtatacatcttgccgccaccagcagagcagttgtccaggaaagatgtcagtctcacttgcctggtcgtgggcttcaaccctggagacatcagtgtggagtggaccagcaatgggcatactgaggagaactacaaggacaccgcaccagtcctggactctgacggttcttacttcatatacagcaagctcgatataaaaacaagcaagtgggagaaaacagattccttctcatgcaacgtgagacacgagggtctgaaaaattactacctgaagaagaccatctcccggtctccgggtaaa

SEQ ID NO: 26 - protein, 214 aa, synthetic construct
DVQITQSPSYLAASPGETITINCRASKRISKNLAWYQEKPGKTIKLLIYSGSTLQSGIPSRFSGSGSGRDFTLIISSLEPEDIAMYYCQQNNEYPLTFGAGTKLELKRADAAPTVSIFPPSSEQLTSGGASVVCFLNNFYPKDINVKWKIDGSERQNGVLNSWTDQDSKDSTYSMSSTLTLTKDEYERHNSYTCEATHKTSTSPIVKSFNRNEC

SEQ ID NO: 27 - protein, 6 aa, synthetic construct
KRISKN

SEQ ID NO: 28 - skipped

SEQ ID NO: 29 - protein, 9 aa, synthetic construct
QQNNEYPLT

SEQ ID NO: 30 - DNA, 642 bp, synthetic construct
  source 1..642: mol_type = other DNA
gatgtccagataacccagtctccatcttatcttgctgcatctcctggagaaaccattactattaattgcagggcaagtaagagaattagcaaaaatttagcctggtatcaggagaaacctgggaaaactattaagcttcttatctactctggatccactttgcaatctggaattccatcaaggttcagtggcagtggatctggtagagatttcactctcatcatcagtagcctggagcctgaagatattgcaatgtattactgtcaacagaataatgaatacccgctcacgttcggtgctgggaccaagctggagctgaaacgggctgatgctgcaccaactgtatccatcttcccaccatccagtgagcagttaacatctggaggtgcctcagtcgtgtgcttcttgaacaacttctaccccaaagacatcaatgtcaagtggaagattgatggcagtgaacgacaaaatggcgtcctgaacagttggactgatcaggacagcaaagacagcacctacagcatgagcagcaccctcacgttgaccaaggacgagtatgaacgacataacagctatacctgtgaggccactcacaagacatcaacttcacccattgtcaagagcttcaacaggaatgagtgt

SEQ ID NO: 31 - protein, 147 aa, synthetic construct
MSARGEGAGQPSTSAQGQPAAPAPQKRGRGRPRKQQQEPTGEPSPKRPRGRPKGSKNKSPSKAAQKKAEATGEKRPRGRPRKWAGVQWYNLGSLQPPPPRFKQFSCLRLLSSWDYRHPPPHPANFCIFSRDRVSPCWPGWSRTPDLR

SEQ ID NO: 32 - protein, 14 aa, synthetic construct
QKRGRGRPRKQQQE

SEQ ID NO: 33 - protein, 9 aa, synthetic construct
IFSRDRVSP

SEQ ID NO: 34 - protein, 19 aa, synthetic construct
RGRPRKWAGVQWYNLGSLQ

SEQ ID NO: 35 - protein, 6 aa, synthetic construct
RGRPRK

SEQ ID NO: 36 - protein, 25 aa, synthetic construct
EVQLQQSGPELVKPGASVRISCKAS

SEQ ID NO: 37 - protein, 17 aa, synthetic construct
MHWVKQSPENSLEWIGE

SEQ ID NO: 38 - protein, 38 aa, synthetic construct
TYNQKFKGKATLTVDKSSITAYMHLKSLTSEDSAVYYC

SEQ ID NO: 39 - protein, 335 aa, synthetic construct
WGQGTTLTVSSAKTTPPSVYPLAPGSAAQTNSMVTLGCLVKGYFPEPVTVTWNSGSLSSGVHTFPAVLQSDLYTLSSSVTVPSSTWPSETVTCNVAHPASSTKVDKKIVPRDCGCKPCICTVPEVSSVFIFPPKPKDVLTITLTPKVTCVVVDISKDDPEVQFSWFVDDVEVHTAQTQPREEQFNSTFRSVSELPIMHQDWLNGKEFKCRVNSAAFPAPIEKTISKTKGRPKAPQVYTIPPPKEQMAKDKVSLTCMITDFFPEDITVEWQWNGQPAENYKNTQPIMDTDGSYFVYSKLNVQKSNWEAGNTFTCSVLHEGLHNHHTEKSLSHSPGK

SEQ ID NO: 40 - protein, 26 aa, synthetic construct
DVSMTQSPLSLPVSLGDQVSISCRSS

SEQ ID NO: 41 - protein, 17 aa, synthetic construct
LEWFLQRPGQSPKLLIY

SEQ ID NO: 42 - protein, 36 aa, synthetic construct
NRFSGVPDRFSGSGSGTDFTLKISRVEAEDLGVYYC

SEQ ID NO: 43 - protein, 117 aa, synthetic construct
FGGGTKLEIKRADAAPTVSIFPPSSEQLTSGGASVVCFLNNFYPKDINVKWKIDGSERQNGVLNSWTDQDSKDSTYSMSSTLTLTKDEYERHNSYTCEATHKTSTSPIVKSFNRNEC

SEQ ID NO: 44 - protein, 25 aa, synthetic construct
QIQLVQSGPELKKPGETVKISCKAS

SEQ ID NO: 45 - protein, 17 aa, synthetic construct
MNWVKQAPGKDLKWMGW

SEQ ID NO: 46 - protein, 37 aa, synthetic construct
YADDFKGRFVFSLETSASTAYLQINNLNNKDTATYFC

SEQ ID NO: 47 - protein, 344 aa, synthetic construct
GTTVTVSSAKTTPPSVYPLAPGCGDTTGSSVTLGCLVKGYFPESVTVTWNSGSLSSSVHTFPALLQSGLYTMSSSVTVPSSTWPSQTVTCSVAHPASSTTVDKKLEPSGPISTINPCPPCKECHKCPAPNLEGGPSVFIFPPNIKDVLMISLTPKVTCVVVDVSEDDPDVRISWFVNNVEVHTAQTQTHREDYNSTIRVVSALPIQHQDWMSGKEFKCKVNNKDLPSPIERTISKIKGLVRAPQVYILPPPAEQLSRKDVSLTCLVVGFNPGDISVEWTSNGHTEENYKDTAPVLDSDGSYFIYSKLDIKTSKWEKTDSFSCNVRHEGLKNYYLKKTISRSPGK

SEQ ID NO: 48 - protein, 26 aa, synthetic construct
DVLMTQTPLSLPVSLGDQASISCRSS

SEQ ID NO: 49 - protein, 17 aa, synthetic construct
LEWYLQKPGQSPKLLIY

SEQ ID NO: 50 - protein, 36 aa, synthetic construct
NRFSGVPDRFSGSGSGTDFTLKITRVEAEDLGVYYC

SEQ ID NO: 51 - protein, 117 aa, synthetic construct; identical to SEQ ID NO: 43

SEQ ID NO: 52 - protein, 25 aa, synthetic construct
EVKLEQSGPELKKPGETVKISCMAS

SEQ ID NO: 53 - protein, 17 aa, synthetic construct
IHWVRQAPGKGLKWMAW

SEQ ID NO: 54 - protein, 38 aa, synthetic construct
TYADDFKGRFAFSLETSASTAYLQINNLENEDTATYYC

SEQ ID NO: 55 - protein, 347 aa, synthetic construct
WGQGTSVTVSSAKTTPPSVYPLAPGCGDTTGSSVTLGCLVKGYFPESVTVTWNSGSLSSSVHTFPALLQSGLYTMSSSVTVPSSTWPSQTVTCSVAHPASSTTVDKKLEPSGPISTINPCPPCKECHKCPAPNLEGGPSVFIFPPNIKDVLMISLTPKVTCVVVDVSEDDPDVRISWFVNNVEVHTAQTQTHREDYNSTIRVVSALPIQHQDWMSGKEFKCKVNNKDLPSPIERTISKIKGLVRAPQVYILPPPAEQLSRKDVSLTCLVVGFNPGDISVEWTSNGHTEENYKDTAPVLDSDGSYFIYSKLDIKTSKWEKTDSFSCNVRHEGLKNYYLKKTISRSPGK

SEQ ID NO: 56 - protein, 26 aa, synthetic construct
DVQITQSPSYLAASPGETITINCRAS

SEQ ID NO: 57 - protein, 17 aa, synthetic construct
LAWYQEKPGKTIKLLIY

SEQ ID NO: 58 - protein, 36 aa, synthetic construct
TLQSGIPSRFSGSGSGRDFTLIISSLEPEDIAMYYC

SEQ ID NO: 59 - protein, 117 aa, synthetic construct
FGAGTKLELKRADAAPTVSIFPPSSEQLTSGGASVVCFLNNFYPKDINVKWKIDGSERQNGVLNSWTDQDSKDSTYSMSSTLTLTKDEYERHNSYTCEATHKTSTSPIVKSFNRNEC